European Patent Application EP 4 596 711 A1, published August 6, 2025. Title: A method for DNA library preparation. Applicant: 国立大学法人九州大学. The sequence listing filed with the application follows.

SEQUENCE LISTING (32 sequences)

SEQ ID NO: 1 - DNA, 33 bp, unidentified
  source 1..33: mol_type = other DNA
agatcggaagagcgtcgtgtagggaaagagtgt

SEQ ID NO: 2 - DNA, 33 bp, unidentified; identical to SEQ ID NO: 1
  source 1..33: mol_type = other DNA

SEQ ID NO: 3 - DNA, 19 bp, unidentified
  source 1..19: mol_type = other DNA
agatcggaagagcgtcgtg

SEQ ID NO: 4 - DNA, 19 bp, unidentified
  source 1..19: mol_type = other DNA
agatcggaagagcgtcgtg

SEQ ID NO: 5 - DNA, 19 bp, unidentified
  source 1..19: mol_type = other DNA
agancggaagagcgtcgtg

SEQ ID NO: 6 - DNA, 50 bp, unidentified
  source 1..50: mol_type = other DNA
gtgactggagttcagacgtgtgctcttccgatccccttattccgatagtg

SEQ ID NO: 7 - DNA, 38 bp, unidentified
  source 1..38: mol_type = other DNA
agggagatcggaagagcacacgtctgaactccagtcac

SEQ ID NO: 8 - DNA, 39 bp, unidentified
  source 1..39: mol_type = other DNA
aagggagatcggaagagcacacgtctgaactccagtcac

SEQ ID NO: 9 - DNA, 11 bp, unidentified
  source 1..11: mol_type = other DNA
cactatcggaa

SEQ ID NO: 10 - DNA, 33 bp, unidentified; identical to SEQ ID NO: 1
  source 1..33: mol_type = other DNA

SEQ ID NO: 11 - DNA, 33 bp, unidentified; identical to SEQ ID NO: 1
  source 1..33: mol_type = other DNA

SEQ ID NO: 12 - DNA, 33 bp, unidentified
  source 1..33: mol_type = other DNA
acactctttccctacacgacgctcttccgatct

SEQ ID NO: 13 - DNA, 34 bp, unidentified
  source 1..34: mol_type = other DNA
acactctttccctacacgacgctcttccgatcta

SEQ ID NO: 14 - DNA, 34 bp, unidentified
  source 1..34: mol_type = other DNA
acactctttccctacacgacgctcttccgatctc

SEQ ID NO: 15 - DNA, 34 bp, unidentified
  source 1..34: mol_type = other DNA
acactctttccctacacgacgctcttccgatctg

SEQ ID NO: 16 - DNA, 34 bp, unidentified
  source 1..34: mol_type = other DNA
acactctttccctacacgacgctcttccgatctt

SEQ ID NO: 17 - DNA, 55 bp, unidentified
  source 1..55: mol_type = other DNA
gatacggcgaccaccgagatctacactctttccctacacgacgctcttccgatct

SEQ ID NO: 18 - DNA, 63 bp, unidentified
  source 1..63: mol_type = other DNA
caagcagaagacggcatacgagatcgtgatgtgactggagttcagacgtgtgctcttccgatc

SEQ ID NO: 19 - DNA, 63 bp, unidentified
  source 1..63: mol_type = other DNA
caagcagaagacggcatacgagatacatcggtgactggagttcagacgtgtgctcttccgatc

SEQ ID NO: 20 - DNA, 63 bp, unidentified
  source 1..63: mol_type = other DNA
caagcagaagacggcatacgagatgcctaagtgactggagttcagacgtgtgctcttccgatc

SEQ ID NO: 21 - DNA, 63 bp, unidentified
  source 1..63: mol_type = other DNA
caagcagaagacggcatacgagattggtcagtgactggagttcagacgtgtgctcttccgatc

SEQ ID NO: 22 - DNA, 63 bp, unidentified
  source 1..63: mol_type = other DNA
caagcagaagacggcatacgagatcactgtgtgactggagttcagacgtgtgctcttccgatc

SEQ ID NO: 23 - DNA, 63 bp, unidentified
  source 1..63: mol_type = other DNA
caagcagaagacggcatacgagatattggcgtgactggagttcagacgtgtgctcttccgatc

SEQ ID NO: 24 - DNA, 63 bp, unidentified
  source 1..63: mol_type = other DNA
caagcagaagacggcatacgagatgatctggtgactggagttcagacgtgtgctcttccgatc

SEQ ID NO: 25 - DNA, 63 bp, unidentified
  source 1..63: mol_type = other DNA
caagcagaagacggcatacgagattcaagtgtgactggagttcagacgtgtgctcttccgatc

SEQ ID NO: 26 - DNA, 63 bp, unidentified
  source 1..63: mol_type = other DNA
caagcagaagacggcatacgagatctgatcgtgactggagttcagacgtgtgctcttccgatc

SEQ ID NO: 27 - DNA, 954 bp, unidentified
  source 1..954: mol_type = other DNA
ggatccatgcgtgcattgttctacaaagacgggaaactttttaccgacaataatttcctgaatccggtaagtgacgacaatccagcgtatgaagttttgcagcacgtgaaaattccgacccatcttaccgatgttgtggtttatgaacaaacgtgggaagaagctctgacccgtctgattttcgttggcagtgattcaaaaggtcgaagacagtacttctacgggaaaatgcatgtccagaatcgcaacgcaaaacgggatcgcatatttgtgcgcgtatataacgtgatgaagcgcatcaattgtttcatcaacaaaaacatcaaaaagagctcaactgattcgaactatcagttagccgtgtttatgctcatggagaccatgttcttcattcgctttggcaaaatgaagtacctcaaagagaatgaaacggtaggcttactgaccttaaagaacaaacacattgaaatcagccctgatgagattgtgatcaaatttgtgggtaaagacaaagtcagccatgaatttgtcgtccacaaatccaatcgcctgtataaaccgctgctgaaactcactgacgattcttccccagaagaatttctgtttaacaaactgtctgaacgtaaggtgtacgagtgcattaagcaattcggtattcgtattaaggatctgcgtacgtatggtgtcaactatacgtttctgtacaacttttggaccaacgtaaagagcatatctcccttacctagtccgaaaaaactgattgcgcttaccatcaaacagacagcggaagttgttggacatacaccgagcatctcaaaacgtgcctatatggctacgactatcctagaaatggtgaaagacaaaaatttcctggatgttgtttcgaaaacgacctttgatgagtttttgtcgattgtcgtggatcatgtgaaaagctccacagatggcgaattc

SEQ ID NO: 28 - DNA, 933 bp, unidentified
  source 1..933: mol_type = other DNA
atgggtcgcggatccatgaaaaagattattttgactattggctgtcctggttctggtaagagtacttgggctcgtgaatttattgctaagaatcccgggttttataatatcaatcgtgatgactatcgccaatctattatggcgcatgaagaacgcgatgagtacaagtataccaaaaagaaagaaggtatcgtaactggtatgcagtttgatacagctaaaagtattctgtacggtggcgattctgttaagggagtaatcatttcagatactaacctgaatcctgaacgtcgcctagcatgggaaacttttgccaaagaatacggctggaaagttgaacataaagtgtttgatgttccttggactgaattggttaaacgtaactcaaaacgcggaactaaagcagtaccaattgatgttttacgttcaatgtataaaagcatgcgagagtatctcggtcttccagtatataatgggactcctggtaaaccaaaagcagttatttttgatgttgatggtacactagctaaaatgaatggtcgtggtccttatgaccttgaaaaatgcgataccgatgttatcaatcctatggttgttgaactgtctaagatgtatgctcttatgggttatcaaatcgtagtcgtttcaggtcgtgaaagtggaactaaagaagacccaacgaaatattatcgtatgacccgtaaatgggttgaggacattgctggcgttccattagttatgcaatgtcagcgcgaacaaggcgatacccgtaaagacgatgtagttaaagaagaaattttctggaaacacattgcaccgcattttgacgtgaaattagctattgatgaccgaactcaagtagttgaaatgtggcgtcgtatcggtgttgaatgctggcaagtcgcttcgggagattttgaattcgagctccgt

SEQ ID NO: 29 - DNA, 34 bp, unidentified
  source 1..34: mol_type = other DNA
agatcggaagagcacacgtctgaactccagtcac

SEQ ID NO: 30 - DNA, 33 bp, unidentified; identical to SEQ ID NO: 1
  source 1..33: mol_type = other DNA

SEQ ID NO: 31 - DNA, 38 bp, unidentified
  source 1..38: mol_type = other DNA
aaggggatcggaagagcacacgtctgaactccagtcac

SEQ ID NO: 32 - DNA, 35 bp, unidentified
  source 1..35: mol_type = other DNA
aaagatcggaagagcgtcgtgtagggaaagagtgt